European Patent Application EP 4 403 578 A1, published July 24, 2024. Title: NEUROPILIN-1 PEPTIDE BASED ANTIBODY, HIGHLITING NEW EPITOPE ASSOCIATED TO GLYCOSAMINOGLYCAN-MODIFIED NEUROPILN-1 AND METHODS OF USE THEREOF. Applicant: THERANOVIR. The sequence listing filed with the application follows.

SEQUENCE LISTING (55 sequences)

SEQ ID NO: 1 - skipped

SEQ ID NO: 2 - protein, 17 aa, synthetic construct
  SITE 1: note = MISC_FEATURE - Y, V or I
  SITE 4: note = MISC_FEATURE - S, Y or P
  SITE 5: note = MISC_FEATURE - G, S or D
  SITE 6: note = MISC_FEATURE - S or G
  SITE 7: note = MISC_FEATURE - S or G
  SITE 8: note = MISC_FEATURE - T or S
  SITE 9: note = MISC_FEATURE - I, K or T
  SITE 10: note = MISC_FEATURE - H, Y or S
  SITE 13: note = MISC_FEATURE - D or Q
  SITE 14: note = MISC_FEATURE - S, K or T
  SITE 15: note = MISC_FEATURE - V or F
  SITE 16: note = MISC_FEATURE - K or Q
XISXXXXXXXYAXXXXG

SEQ ID NO: 3 - protein, 13 aa, Mus musculus
RHYGSSRYWYFDV

SEQ ID NO: 4 - protein, 11 aa, synthetic construct
  SITE 1: note = MISC_FEATURE - K or R
  SITE 5: note = MISC_FEATURE - D or S
  SITE 6: note = MISC_FEATURE - I or V
  SITE 7: note = MISC_FEATURE - K or S
  SITE 9: note = MISC_FEATURE - Y or W
  SITE 11: note = MISC_FEATURE - S or A
XASQXXXSXLX

SEQ ID NO: 5 - skipped

SEQ ID NO: 6 - protein, 9 aa, synthetic construct
  SITE 1: note = synthetic - L or Q
  SITE 4: note = synthetic - G or S
  SITE 5: note = synthetic - E or S
  SITE 7: note = synthetic - P or S
XQYXXSXYT

SEQ ID NO: 7 - protein, 5 aa, Mus musculus
SFGMH

SEQ ID NO: 8 - protein, 17 aa, Mus musculus
YISSGSSTIHYADTVKG

SEQ ID NO: 9 - protein, 13 aa, Mus musculus
RHYGSSRYWYFDV

SEQ ID NO: 10 - protein, 11 aa, Mus musculus
KASQDIKSYLS

SEQ ID NO: 11 - protein, 7 aa, Mus musculus
YATSLAG

SEQ ID NO: 12 - protein, 9 aa, Mus musculus
LQYGESPYT

SEQ ID NO: 13 - protein, 122 aa, synthetic construct
EVQLVESGGGLVQPGGSLRLSCAASGFTFSSFGMHWVRQAPGKGLEWVAYISSGSSTIHYADSVKGRFTISRDNAKNSLYLQMNSLRAEDTAMYYCARRHYGSSRYWYFDVWGQGTTVTVSS

SEQ ID NO: 14 - protein, 122 aa, synthetic construct
EVQLVESGGGLVQPGGSLRLSCAASGFTFSSYSMHWVRQAPGKGLEWVSYISSGSSTIHYADSVKGRFTISRDNAKNSLYLQMNSLRAEDTAVYYCARRHYGSSRYWYFDVWGQGTTVTVSS

SEQ ID NO: 15 - protein, 122 aa, synthetic construct
EVQLVESGGGLVQPGGSLRLSCAASGFTFSSYSMHWVRQAPGKGLEWVSYISSSSSTIYYADSVKGRFTISRDNAKNSLYLQMNSLRAEDTAVYYCARRHYGSSRYWYFDVWGQGTTVTVSS

SEQ ID NO: 16 - protein, 122 aa, synthetic construct
QVQLVESGGGVVQPGGSLRLSCAASGFTFSSFGMHWVRQAPGKGLEWVAYISSGSSTIHYADSVKGRFTISRDNSKNTLYLQMNSLRAEDTAMYYCARRHYGSSRYWYFDVWGQGTTVTVSS

SEQ ID NO: 17 - protein, 122 aa, synthetic construct
QVQLVESGGGVVQPGRSLRLSCAASGFTFSSYGMHWVRQAPGKGLEWVAYISSGGSTKHYADSVKGRFTISRDNSKNTLYLQMNSLRAEDTAVYYCARRHYGSSRYWYFDVWGQGTTVTVSS

SEQ ID NO: 18 - protein, 122 aa, synthetic construct
QVQLVESGGGVVQPGRSLRLSCAASGFTFSSYGMHWVRQAPGKGLEWVAVISYDGSTKYYADSVKGRFTISRDNSKNTLYLQMNSLRAEDTAVYYCARRHYGSSRYWYFDVWGQGTTVTVSS

SEQ ID NO: 19 - protein, 122 aa, synthetic construct
QVQLVQSGAEVKKPGASVKVSCKASGYTFTSFGMHWVRQAPGQGLEWMGYISSSSSTIHYAQKVKGRFTITRDNSTNTLYLEMSSLRSEDTAMYYCARRHYGSSRYWYFDVWGQGTTVTVSS

SEQ ID NO: 20 - protein, 122 aa, synthetic construct
QVQLVQSGAEVKKPGASVKVSCKASGYTFTSYGMHWVRQAPGQGLEWMGYISSSGSSTHYAQKFQGRFTMTRDTSTSTVYMELSSLRSEDTAVYYCARRHYGSSRYWYFDVWGQGTTVTVSS

SEQ ID NO: 21 - protein, 122 aa, synthetic construct
QVQLVQSGAEVKKPGASVKVSCKASGYTFTSYYMHWVRQAPGQGLEWMGIISPSGGSTSYAQKFQGRVTMTRDTSTSTVYMELSSLRSEDTAVYYCARRHYGSSRYWYFDVWGQGTTVTVSS

SEQ ID NO: 22 - protein, 107 aa, synthetic construct
DIQMTQSPSTLSASVGDRVTITCRASQDIKSYLSWYQQKPGKAPKTLIYYATSLAGGVPSRFSGSGSGQEYTLTISSLQPDDFATYYCLQYGESPYTFGQGTKLEIK

SEQ ID NO: 23 - protein, 107 aa, synthetic construct
DIQMTQSPSTLSASVGDRVTITCRASQSIKSYLAWYQQKPGKAPKLLIYYASSLASGVPSRFSGSGSGTEFTLTISSLQPDDFATYYCQQYGESSYTFGQGTKLEIK

SEQ ID NO: 24 - protein, 107 aa, synthetic construct
DIQMTQSPSTLSASVGDRVTITCRASQSISSWLAWYQQKPGKAPKLLIYYASSLESGVPSRFSGSGSGTEFTLTISSLQPDDFATYYCQQYGSSSYTFGQGTKLEIK

SEQ ID NO: 25 - protein, 107 aa, synthetic construct
EIVMTQSPATLSLSPGERATLSCRASQDIKSYLSWYQQKPGQAPRTLIYYATSLAGGIPARFSGSGSGQDYTLTISSLEPEDFAVYYCLQYGESPYTFGQGTKLEIK

SEQ ID NO: 26 - protein, 107 aa, synthetic construct
EIVLTQSPATLSLSPGERATLSCRASQSVKSYLAWYQQKPGQAPRLLIYYASSRATGIPARFSGSGSGTDFTLTISSLEPEDFAVYYCQQYSESPYTFGQGTKLEIK

SEQ ID NO: 27 - protein, 107 aa, synthetic construct
EIVLTQSPATLSLSPGERATLSCRASQSVSSYLAWYQQKPGQAPRLLIYDASSRATGIPARFSGSGSGTDFTLTISSLEPEDFAVYYCQQYSESPYTFGQGTKLEIK

SEQ ID NO: 28 - skipped

SEQ ID NO: 29 - protein, 17 aa, synthetic construct
  SITE 1: note = MISC_FEATURE - Y or V
  SITE 4: note = MISC_FEATURE - S or Y
  SITE 5: note = MISC_FEATURE - S or G
  SITE 6: note = MISC_FEATURE - S or G
  SITE 9: note = MISC_FEATURE - I or K
  SITE 14: note = MISC_FEATURE - T or S
  SITE 14: note = MISC_FEATURE - T or S
XISXXXSTXYYADXVKG

SEQ ID NO: 30 - protein, 13 aa, synthetic construct
RHYGRSRYWYFDV

SEQ ID NO: 31 - protein, 11 aa, synthetic construct
  SITE 1: note = MISC_FEATURE - K or R
  SITE 5: note = MISC_FEATURE - D or S
  SITE 6: note = MISC_FEATURE - I or V
  SITE 7: note = MISC_FEATURE - K or S
  SITE 11: note = MISC_FEATURE - S or A
XASQXXXSYLX

SEQ ID NO: 32 - skipped

SEQ ID NO: 33 - protein, 9 aa, synthetic construct
  SITE 1: note = MISC_FEATURE - L or Q
  SITE 7: note = MISC_FEATURE - P or S
XQYGESXYT

SEQ ID NO: 34 - protein, 5 aa, synthetic construct
SFGMH

SEQ ID NO: 35 - protein, 17 aa, synthetic construct
YISSGSSTIYYADTVKG

SEQ ID NO: 36 - protein, 13 aa, synthetic construct
RHYGRSRYWYFDV

SEQ ID NO: 37 - protein, 11 aa, Mus musculus
KASQDIKSYLS

SEQ ID NO: 38 - protein, 7 aa, Mus musculus
YATSLAD

SEQ ID NO: 39 - protein, 9 aa, synthetic construct
LQYGESPYT

SEQ ID NO: 40 - protein, 122 aa, synthetic construct
EVQLVESGGGLVQPGGSLRLSCAASGFTFSSFGMHWVRQAPGKGLEWVAYISSGSSTIYYADTVKGRFTISRDNPKNSLYLQMTSLRAEDTAVYYCTRRHYGRSRYWYFDVWGQGTTVTVSS

SEQ ID NO: 41 - protein, 122 aa, synthetic construct
EVQLVESGGGLVQPGGSLRLSCAASGFTFSSYSMHWVRQAPGKGLEWVSYISSSSSTIYYADSVKGRFTISRDNAKNSLYLQMTSLRAEDTAVYYCARRHYGRSRYWYFDVWGQGTTVTVSS

SEQ ID NO: 42 - protein, 122 aa, synthetic construct
QVQLVESGGGLVKPGGSLRLSCAASGFTFSSFGMHWIRQAPGKGLEWVAYISSGSSTIYYADTVKGRFTISRDNPKNSLYLQMTSLRAEDTAVYYCTRRHYGRSRYWYFDVWGQGTTVTVSS

SEQ ID NO: 43 - protein, 122 aa, synthetic construct
QVQLVESGGGLVKPGGSLRLSCAASGFTFSSYGMHWIRQAPGKGLEWVSYISSSGSTIYYADSVKGRFTISRDNAKNSLYLQMTSLRAEDTAVYYCARRHYGRSRYWYFDVWGQGTTVTVSS

SEQ ID NO: 44 - protein, 122 aa, synthetic construct
QVQLVESGGGLVKPGGSLRLSCAASGFTFSSYYMSWIRQAPGKGLEWVSYISSSGSTIYYADSVKGRFTISRDNAKNSLYLQMTSLRAEDTAVYYCARRHYGRSRYWYFDVWGQGTTVTVSS

SEQ ID NO: 45 - protein, 122 aa, synthetic construct
QVQLVESGGGVVQPGRSLRLSCAASGFTFSSFGMHWVRQAPGKGLEWVAYISSGSSTIYYADTVKGRFTISRDNPKNTLYLQMTSLRAEDTAVYYCTRRHYGRSRYWYFDVWGQGTTVTVSS

SEQ ID NO: 46 - protein, 122 aa, synthetic construct
QVQLVESGGGVVQPGRSLRLSCAASGFTFSSYAMHWVRQAPGKGLEWVAYISSGGSTIYYADSVKGRFTISRDNSKNTLYLQMTSLRAEDTAVYYCARRHYGRSRYWYFDVWGQGTTVTVSS

SEQ ID NO: 47 - protein, 122 aa, synthetic construct
QVQLVESGGGVVQPGRSLRLSCAASGFTFSSYAMHWVRQAPGKGLEWVAVISYGGSTKYYADSVKGRFTISRDNSKNTLYLQMTSLRAEDTAVYYCARRHYGRSRYWYFDVWGQGTTVTVSS

SEQ ID NO: 48 - protein, 107 aa, synthetic construct
EIQMTQSPSTLSASVGERVTITCRASQDIKSYLSWYQQKPGKAPKTLIYYATSLADGVPSRFSGSGSGQEYTLTISSLQPEDFATYYCLQYGESPYTFGQGTKLEIK

SEQ ID NO: 49 - protein, 107 aa, synthetic construct
EIQMTQSPSTLSASVGERVTITCRASQDIKSYLAWYQQKPGKAPKLLIYYASSLASGVPSRFSGSGSGTEFTLTISSLQPEDFATYYCLQYGESSYTFGQGTKLEIK

SEQ ID NO: 50 - protein, 107 aa, synthetic construct
EIQMTQSPSTLSASVGERVTITCRASQSISSYLAWYQQKPGKAPKLLIYYASSLESGVPSRFSGSGSGTEFTLTISSLQPEDFATYYCQQYGESSYTFGQGTKLEIK

SEQ ID NO: 51 - protein, 107 aa, synthetic construct
EIVMTQSPGTLSLSPGERATLSCRASQDIKSYLSWYQQKPGQAPRTLIYYATSLADGIPSRFSGSGSGQEYTLTISRLEPEDFAVYYCLQYGESPYTFGQGTKLEIK

SEQ ID NO: 52 - protein, 107 aa, synthetic construct
EIVLTQSPGTLSLSPGERATLSCRASQDVKSYLAWYQQKPGQAPRLLIYYASSRATGIPSRFSGSGSGTEFTLTISRLEPEDFAVYYCLQYGESPYTFGQGTKLEIK

SEQ ID NO: 53 - protein, 107 aa, synthetic construct
EIVLTQSPGTLSLSPGERATLSCRASQSVSSYLAWYQQKPGQAPRLLIYGASSRATGIPSRFSGSGSGTEFTLTISRLEPEDFAVYYCQQYGESPYTFGQGTKLEIK

SEQ ID NO: 54 - protein, 24 aa, synthetic construct
EGNKPVLFQGNTNPTDVVVAVFPK

SEQ ID NO: 55 - protein, 19 aa, synthetic construct
EGNKPVLFQGNTNPTDVVC